European Patent Specification EP 3 997 220 B1, published September 10, 2025. Title: NOVEL ESTERASES AND USES THEREOF. Applicant: CARBIOS. The sequence listing filed with the application follows.

SEQUENCE LISTING (1 sequence)

SEQ ID NO: 1 - protein, 259 aa, ARTIFICIAL SEQUNECE
  parent esterase
MANPYERGPDPTESSIEAVRGPFAVAQTTVSRLQADGFGGGTIYYPTDTSQGTFGAVAISPGFTAGQESIAWLGPRIASQGFVVITIDTITRLDQPDSRGRQLQAALDHLRTNSVVRNRIDPNRMAVMGHSMGGGGALSAAANNTSLEAAIPLQGWHTRKNWSSVRTPTLVVGAQLDTIAPVSSHSEAFYNSLPSDLDKAYMELRGASHLVSNTPDTTTAKYSIAWLKRFVDDDLRYEQFLCPAPDDFAISEYRSTCPF